European Patent Application EP 4 209 503 A1, published July 12, 2023. Title: IL-2 MUTANT AND APPLICATION THEREOF. Applicant: Jiangsu Simcere Pharmaceutrical Co.Ltd. The sequence listing filed with the application follows.

SEQUENCE LISTING (60 sequences)

SEQ ID NO: 1 - protein, 133 aa, Homo sapiens
APTSSSTKKTQLQLEHLLLDLQMILNGINNYKNPKLTRMLTFKFYMPKKATELKHLQCLEEELKPLEEVLNLAQSKNFHLRPRDLISNINVIVLELKGSETTFMCEYADETATIVEFLNRWITFAQSIISTLT

SEQ ID NO: 2 - protein, 133 aa, Artificial Sequence
APTSSSTKKTQLQLEHLLLDLQMILNGINNVKNPKLTRMLTFKFYMPKKATELKHLQCLEEELKPLEEVLNLLQSKNFQLRPRDLISNINVIVLELKGSETTFMCEYADETATIVEFLNRWITFAQSIISTLT

SEQ ID NO: 3 - protein, 133 aa, Artificial Sequence
APTSSSTKKTQLLLEHLLLDLQMILNGINNYKNPKLTRMLTFKFYMPKKATELKHLQCLEEELKPLEEVLNLAQSKNFHLRPRDLISNINVIVLELKGSETTFMCEYADETATIVEFLNRWITFAQSIISTLT

SEQ ID NO: 4 - protein, 133 aa, Artificial Sequence
APTSSSTKKTQLQLEHLLLDLQMILNGINNYKNPKLTRMLTFKFYMPKKATELKHLQCLEEELKPLEEVLNLAQSKNFHLRPRDLISNINVIVLELKGSETTFMCEYADETATIVEFLNFWITFAQSIISTLT

SEQ ID NO: 5 - protein, 133 aa, Artificial Sequence
APTSSSTKKTQLQLEHLILDLQMILNGINNYKNPKLTRMLTFKFYMPKKATELKHLQCLEEELKPLEEVLNLAQSKNFHLRPRDLISNINAIVLELKGSETTFMCEYADETATIVEWLNRWITFAQSIISTLT

SEQ ID NO: 6 - protein, 133 aa, Artificial Sequence
APTSSSTKKTQLQLEHLILDLQMILNGINNYKNPKLTRMLTFKFYMPKKATELKHLQCLEEELKPLEEVLNLAQSKNFHLRPRDLISNLNVIILELKGSETTFMCEYADETATIVEFLNRWITFAQSIISTLT

SEQ ID NO: 7 - protein, 133 aa, Artificial Sequence
APTSSSTKKTQLQLEHLLLDLQMILNWINNYKNPKLTRMLTFKFYMPKKATELKHLQCLEEELKPLEEVLNLAQSKNFHLRPRDLISNINVIVLELKGSETTFMCEYADETATIVEFLNFWITFAQSIISTLT

SEQ ID NO: 8 - protein, 133 aa, Artificial Sequence
APTSSSTKKTQLQLEHLLLDLQMILNGINNYKNPKLTRMLTFKFYMPKKATELKHLQCLEEELKPLEEVLNLAQSKNFHLRLRDLISNINVIVLELKGSETTFMCEYADETATIVEFLNFWITFAQSIISTLT

SEQ ID NO: 9 - protein, 133 aa, Artificial Sequence
APTSSSTKKTQLQLEHLLLDLQMILNGINNYKNPKLTRMLTFKFYMPKKATELKHLQCLEEELKPLEEVLNLAQSKNFHLRPRDLISNIYVIVLELKGSETTFMCEYADETATIVEFLNFWITFAQSIISTLT

SEQ ID NO: 10 - protein, 15 aa, Artificial Sequence
GGGGSGGGGSGGGGS

SEQ ID NO: 11 - protein, 232 aa, Artificial Sequence
EPKSSDKTHTCPPCPAPELLGGPSVFLFPPKPKDTLMISRTPEVTCVVVDVSHEDPEVKFNWYVDGVEVHNAKTKPREEQYGSTYRVVSVLTVLHQDWLNGKEYKCKVSNKALPAPIEKTISKAKGQPREPQVYTLPPSRDELTKNQVSLTCLVKGFYPSDIAVEWESNGQPENNYKTTPPVLDSDGSFFLYSKLTVDKSRWQQGNVFSCSVMHEALHNHYTQKSLSLSPGK

SEQ ID NO: 12 - protein, 380 aa, Artificial Sequence
APTSSSTKKTQLQLEHLLLDLQMILNGINNYKNPKLTRMLTFKFYMPKKATELKHLQCLEEELKPLEEVLNLAQSKNFHLRPRDLISNINVIVLELKGSETTFMCEYADETATIVEFLNRWITFAQSIISTLTGGGGSGGGGSGGGGSEPKSSDKTHTCPPCPAPELLGGPSVFLFPPKPKDTLMISRTPEVTCVVVDVSHEDPEVKFNWYVDGVEVHNAKTKPREEQYGSTYRVVSVLTVLHQDWLNGKEYKCKVSNKALPAPIEKTISKAKGQPREPQVYTLPPSRDELTKNQVSLTCLVKGFYPSDIAVEWESNGQPENNYKTTPPVLDSDGSFFLYSKLTVDKSRWQQGNVFSCSVMHEALHNHYTQKSLSLSPGK

SEQ ID NO: 13 - protein, 380 aa, Artificial Sequence
APTSSSTKKTQLQLEHLLLDLQMILNGINNVKNPKLTRMLTFKFYMPKKATELKHLQCLEEELKPLEEVLNLLQSKNFQLRPRDLISNINVIVLELKGSETTFMCEYADETATIVEFLNRWITFAQSIISTLTGGGGSGGGGSGGGGSEPKSSDKTHTCPPCPAPELLGGPSVFLFPPKPKDTLMISRTPEVTCVVVDVSHEDPEVKFNWYVDGVEVHNAKTKPREEQYGSTYRVVSVLTVLHQDWLNGKEYKCKVSNKALPAPIEKTISKAKGQPREPQVYTLPPSRDELTKNQVSLTCLVKGFYPSDIAVEWESNGQPENNYKTTPPVLDSDGSFFLYSKLTVDKSRWQQGNVFSCSVMHEALHNHYTQKSLSLSPGK

SEQ ID NO: 14 - protein, 380 aa, Artificial Sequence
APTSSSTKKTQLLLEHLLLDLQMILNGINNYKNPKLTRMLTFKFYMPKKATELKHLQCLEEELKPLEEVLNLAQSKNFHLRPRDLISNINVIVLELKGSETTFMCEYADETATIVEFLNRWITFAQSIISTLTGGGGSGGGGSGGGGSEPKSSDKTHTCPPCPAPELLGGPSVFLFPPKPKDTLMISRTPEVTCVVVDVSHEDPEVKFNWYVDGVEVHNAKTKPREEQYGSTYRVVSVLTVLHQDWLNGKEYKCKVSNKALPAPIEKTISKAKGQPREPQVYTLPPSRDELTKNQVSLTCLVKGFYPSDIAVEWESNGQPENNYKTTPPVLDSDGSFFLYSKLTVDKSRWQQGNVFSCSVMHEALHNHYTQKSLSLSPGK

SEQ ID NO: 15 - protein, 380 aa, Artificial Sequence
APTSSSTKKTQLQLEHLLLDLQMILNGINNYKNPKLTRMLTFKFYMPKKATELKHLQCLEEELKPLEEVLNLAQSKNFHLRPRDLISNINVIVLELKGSETTFMCEYADETATIVEFLNFWITFAQSIISTLTGGGGSGGGGSGGGGSEPKSSDKTHTCPPCPAPELLGGPSVFLFPPKPKDTLMISRTPEVTCVVVDVSHEDPEVKFNWYVDGVEVHNAKTKPREEQYGSTYRVVSVLTVLHQDWLNGKEYKCKVSNKALPAPIEKTISKAKGQPREPQVYTLPPSRDELTKNQVSLTCLVKGFYPSDIAVEWESNGQPENNYKTTPPVLDSDGSFFLYSKLTVDKSRWQQGNVFSCSVMHEALHNHYTQKSLSLSPGK

SEQ ID NO: 16 - protein, 380 aa, Artificial Sequence
APTSSSTKKTQLQLEHLILDLQMILNGINNYKNPKLTRMLTFKFYMPKKATELKHLQCLEEELKPLEEVLNLAQSKNFHLRPRDLISNINAIVLELKGSETTFMCEYADETATIVEWLNRWITFAQSIISTLTGGGGSGGGGSGGGGSEPKSSDKTHTCPPCPAPELLGGPSVFLFPPKPKDTLMISRTPEVTCVVVDVSHEDPEVKFNWYVDGVEVHNAKTKPREEQYGSTYRVVSVLTVLHQDWLNGKEYKCKVSNKALPAPIEKTISKAKGQPREPQVYTLPPSRDELTKNQVSLTCLVKGFYPSDIAVEWESNGQPENNYKTTPPVLDSDGSFFLYSKLTVDKSRWQQGNVFSCSVMHEALHNHYTQKSLSLSPGK

SEQ ID NO: 17 - protein, 380 aa, Artificial Sequence
APTSSSTKKTQLQLEHLILDLQMILNGINNYKNPKLTRMLTFKFYMPKKATELKHLQCLEEELKPLEEVLNLAQSKNFHLRPRDLISNLNVIILELKGSETTFMCEYADETATIVEFLNRWITFAQSIISTLTGGGGSGGGGSGGGGSEPKSSDKTHTCPPCPAPELLGGPSVFLFPPKPKDTLMISRTPEVTCVVVDVSHEDPEVKFNWYVDGVEVHNAKTKPREEQYGSTYRVVSVLTVLHQDWLNGKEYKCKVSNKALPAPIEKTISKAKGQPREPQVYTLPPSRDELTKNQVSLTCLVKGFYPSDIAVEWESNGQPENNYKTTPPVLDSDGSFFLYSKLTVDKSRWQQGNVFSCSVMHEALHNHYTQKSLSLSPGK

SEQ ID NO: 18 - protein, 380 aa, Artificial Sequence
APTSSSTKKTQLQLEHLLLDLQMILNWINNYKNPKLTRMLTFKFYMPKKATELKHLQCLEEELKPLEEVLNLAQSKNFHLRPRDLISNINVIVLELKGSETTFMCEYADETATIVEFLNFWITFAQSIISTLTGGGGSGGGGSGGGGSEPKSSDKTHTCPPCPAPELLGGPSVFLFPPKPKDTLMISRTPEVTCVVVDVSHEDPEVKFNWYVDGVEVHNAKTKPREEQYGSTYRVVSVLTVLHQDWLNGKEYKCKVSNKALPAPIEKTISKAKGQPREPQVYTLPPSRDELTKNQVSLTCLVKGFYPSDIAVEWESNGQPENNYKTTPPVLDSDGSFFLYSKLTVDKSRWQQGNVFSCSVMHEALHNHYTQKSLSLSPGK

SEQ ID NO: 19 - protein, 380 aa, Artificial Sequence
APTSSSTKKTQLQLEHLLLDLQMILNGINNYKNPKLTRMLTFKFYMPKKATELKHLQCLEEELKPLEEVLNLAQSKNFHLRLRDLISNINVIVLELKGSETTFMCEYADETATIVEFLNFWITFAQSIISTLTGGGGSGGGGSGGGGSEPKSSDKTHTCPPCPAPELLGGPSVFLFPPKPKDTLMISRTPEVTCVVVDVSHEDPEVKFNWYVDGVEVHNAKTKPREEQYGSTYRVVSVLTVLHQDWLNGKEYKCKVSNKALPAPIEKTISKAKGQPREPQVYTLPPSRDELTKNQVSLTCLVKGFYPSDIAVEWESNGQPENNYKTTPPVLDSDGSFFLYSKLTVDKSRWQQGNVFSCSVMHEALHNHYTQKSLSLSPGK

SEQ ID NO: 20 - protein, 380 aa, Artificial Sequence
APTSSSTKKTQLQLEHLLLDLQMILNGINNYKNPKLTRMLTFKFYMPKKATELKHLQCLEEELKPLEEVLNLAQSKNFHLRPRDLISNIYVIVLELKGSETTFMCEYADETATIVEFLNFWITFAQSIISTLTGGGGSGGGGSGGGGSEPKSSDKTHTCPPCPAPELLGGPSVFLFPPKPKDTLMISRTPEVTCVVVDVSHEDPEVKFNWYVDGVEVHNAKTKPREEQYGSTYRVVSVLTVLHQDWLNGKEYKCKVSNKALPAPIEKTISKAKGQPREPQVYTLPPSRDELTKNQVSLTCLVKGFYPSDIAVEWESNGQPENNYKTTPPVLDSDGSFFLYSKLTVDKSRWQQGNVFSCSVMHEALHNHYTQKSLSLSPGK

SEQ ID NO: 21 - protein, 133 aa, Artificial Sequence
APTSSSTKKTQLQLEELLLDLQMILNGINNYKNPKLTRMLTFKFYMPKKATELKHLQCLEEELKPLEEVLNLAQSKNFHLRPRDLISNINVIVLELKGSETTFMCEYADETATIVEFLNRWITFAQSIISTLT

SEQ ID NO: 22 - protein, 133 aa, Artificial Sequence
APTSSSTKKTQLQLEELLLDLQMILNGINNVKNPKLTRMLTFKFYMPKKATELKHLQCLEEELKPLEEVLNLLQSKNFQLRPRDLISNINVIVLELKGSETTFMCEYADETATIVEFLNRWITFAQSIISTLT

SEQ ID NO: 23 - protein, 133 aa, Artificial Sequence
APTSSSTKKTQLQLEELLLDLQMILNGINNYKNPKLTRMLTFKFYMPKKATELKHLQCLEEELKPLEEVLNLAQSKNFHLRPRDLISNINVIVLELKGSETTFMCEYADETATIVEFLNFWITFAQSIISTLT

SEQ ID NO: 24 - protein, 133 aa, Artificial Sequence
APTSSSTKKTQLQLEELILDLQMILNGINNYKNPKLTRMLTFKFYMPKKATELKHLQCLEEELKPLEEVLNLAQSKNFHLRPRDLISNINAIVLELKGSETTFMCEYADETATIVEWLNRWITFAQSIISTLT

SEQ ID NO: 25 - protein, 133 aa, Artificial Sequence
APTSSSTKKTQLQLEELILDLQMILNGINNYKNPKLTRMLTFKFYMPKKATELKHLQCLEEELKPLEEVLNLAQSKNFHLRPRDLISNLNVIILELKGSETTFMCEYADETATIVEFLNRWITFAQSIISTLT

SEQ ID NO: 26 - protein, 133 aa, Artificial Sequence
APTSSSTKKTQLQLEELLLDLQMILNWINNYKNPKLTRMLTFKFYMPKKATELKHLQCLEEELKPLEEVLNLAQSKNFHLRPRDLISNINVIVLELKGSETTFMCEYADETATIVEFLNFWITFAQSIISTLT

SEQ ID NO: 27 - protein, 133 aa, Artificial Sequence
APTSSSTKKTQLQLEELLLDLQMILNGINNYKNPKLTRMLTFKFYMPKKATELKHLQCLEEELKPLEEVLNLAQSKNFHLRLRDLISNINVIVLELKGSETTFMCEYADETATIVEFLNFWITFAQSIISTLT

SEQ ID NO: 28 - protein, 133 aa, Artificial Sequence
APTSSSTKKTQLQLEHLLLALQMILNGINNYKNPKLTRMLTFKFYMPKKATELKHLQCLEEELKPLEEVLNLAQSKNFHLRPRDLISNINVIVLELKGSETTFMCEYADETATIVEFLNRWITFAQSIISTLT

SEQ ID NO: 29 - protein, 133 aa, Artificial Sequence
APTSSSTKKTQLQLEHLLLALQMILNGINNVKNPKLTRMLTFKFYMPKKATELKHLQCLEEELKPLEEVLNLLQSKNFQLRPRDLISNINVIVLELKGSETTFMCEYADETATIVEFLNRWITFAQSIISTLT

SEQ ID NO: 30 - protein, 133 aa, Artificial Sequence
APTSSSTKKTQLQLEHLLLALQMILNGINNYKNPKLTRMLTFKFYMPKKATELKHLQCLEEELKPLEEVLNLAQSKNFHLRPRDLISNINVIVLELKGSETTFMCEYADETATIVEFLNFWITFAQSIISTLT

SEQ ID NO: 31 - protein, 133 aa, Artificial Sequence
APTSSSTKKTQLQLEHLLLDLQMILNGINNYKNPKLTRMLTFKFYMPKKATELKHLQCLEEELKPLEEVLNLAQSKNFHLRPRDLISNINRIVLELKGSETTFMCEYADETATIVEFLNRWITFAQSIISTLT

SEQ ID NO: 32 - protein, 133 aa, Artificial Sequence
APTSSSTKKTQLQLEHLLLDLQMILNGINNVKNPKLTRMLTFKFYMPKKATELKHLQCLEEELKPLEEVLNLLQSKNFQLRPRDLISNINRIVLELKGSETTFMCEYADETATIVEFLNRWITFAQSIISTLT

SEQ ID NO: 33 - protein, 133 aa, Artificial Sequence
APTSSSTKKTQLLLEHLLLDLQMILNGINNYKNPKLTRMLTFKFYMPKKATELKHLQCLEEELKPLEEVLNLAQSKNFHLRPRDLISNINRIVLELKGSETTFMCEYADETATIVEFLNRWITFAQSIISTLT

SEQ ID NO: 34 - protein, 133 aa, Artificial Sequence
APTSSSTKKTQLQLEHLLLDLQMILNGINNYKNPKLTRMLTFKFYMPKKATELKHLQCLEEELKPLEEVLNLAQSKNFHLRPRDLISNINRIVLELKGSETTFMCEYADETATIVEFLNFWITFAQSIISTLT

SEQ ID NO: 35 - protein, 133 aa, Artificial Sequence
APTSSSTKKTQLQLEHLILDLQMILNGINNYKNPKLTRMLTFKFYMPKKATELKHLQCLEEELKPLEEVLNLAQSKNFHLRPRDLISNLNRIILELKGSETTFMCEYADETATIVEFLNRWITFAQSIISTLT

SEQ ID NO: 36 - protein, 133 aa, Artificial Sequence
APTSSSTKKTQLQLEELLLDLQMILNGINNYKNPKLTRMLTFKFYMPKKATELKHLQCLEEELKPLEEVLNLAQSKNFHLRPRDLISNINRIVLELKGSETTFMCEYADETATIVEFLNRWITFAQSIISTLT

SEQ ID NO: 37 - protein, 133 aa, Artificial Sequence
APTSSSTKKTQLQLEELLLDLQMILNGINNVKNPKLTRMLTFKFYMPKKATELKHLQCLEEELKPLEEVLNLLQSKNFQLRPRDLISNINRIVLELKGSETTFMCEYADETATIVEFLNRWITFAQSIISTLT

SEQ ID NO: 38 - protein, 133 aa, Artificial Sequence
APTSSSTKKTQLQLEELILDLQMILNGINNYKNPKLTRMLTFKFYMPKKATELKHLQCLEEELKPLEEVLNLAQSKNFHLRPRDLISNLNRIILELKGSETTFMCEYADETATIVEFLNRWITFAQSIISTLT

SEQ ID NO: 39 - protein, 380 aa, Artificial Sequence
APTSSSTKKTQLQLEELLLDLQMILNGINNYKNPKLTRMLTFKFYMPKKATELKHLQCLEEELKPLEEVLNLAQSKNFHLRPRDLISNINVIVLELKGSETTFMCEYADETATIVEFLNRWITFAQSIISTLTGGGGSGGGGSGGGGSEPKSSDKTHTCPPCPAPELLGGPSVFLFPPKPKDTLMISRTPEVTCVVVDVSHEDPEVKFNWYVDGVEVHNAKTKPREEQYGSTYRVVSVLTVLHQDWLNGKEYKCKVSNKALPAPIEKTISKAKGQPREPQVYTLPPSRDELTKNQVSLTCLVKGFYPSDIAVEWESNGQPENNYKTTPPVLDSDGSFFLYSKLTVDKSRWQQGNVFSCSVMHEALHNHYTQKSLSLSPGK

SEQ ID NO: 40 - protein, 380 aa, Artificial Sequence
APTSSSTKKTQLQLEELLLDLQMILNGINNVKNPKLTRMLTFKFYMPKKATELKHLQCLEEELKPLEEVLNLLQSKNFQLRPRDLISNINVIVLELKGSETTFMCEYADETATIVEFLNRWITFAQSIISTLTGGGGSGGGGSGGGGSEPKSSDKTHTCPPCPAPELLGGPSVFLFPPKPKDTLMISRTPEVTCVVVDVSHEDPEVKFNWYVDGVEVHNAKTKPREEQYGSTYRVVSVLTVLHQDWLNGKEYKCKVSNKALPAPIEKTISKAKGQPREPQVYTLPPSRDELTKNQVSLTCLVKGFYPSDIAVEWESNGQPENNYKTTPPVLDSDGSFFLYSKLTVDKSRWQQGNVFSCSVMHEALHNHYTQKSLSLSPGK

SEQ ID NO: 41 - protein, 380 aa, Artificial Sequence
APTSSSTKKTQLQLEELLLDLQMILNGINNYKNPKLTRMLTFKFYMPKKATELKHLQCLEEELKPLEEVLNLAQSKNFHLRPRDLISNINVIVLELKGSETTFMCEYADETATIVEFLNFWITFAQSIISTLTGGGGSGGGGSGGGGSEPKSSDKTHTCPPCPAPELLGGPSVFLFPPKPKDTLMISRTPEVTCVVVDVSHEDPEVKFNWYVDGVEVHNAKTKPREEQYGSTYRVVSVLTVLHQDWLNGKEYKCKVSNKALPAPIEKTISKAKGQPREPQVYTLPPSRDELTKNQVSLTCLVKGFYPSDIAVEWESNGQPENNYKTTPPVLDSDGSFFLYSKLTVDKSRWQQGNVFSCSVMHEALHNHYTQKSLSLSPGK

SEQ ID NO: 42 - protein, 380 aa, Artificial Sequence
APTSSSTKKTQLQLEELILDLQMILNGINNYKNPKLTRMLTFKFYMPKKATELKHLQCLEEELKPLEEVLNLAQSKNFHLRPRDLISNINAIVLELKGSETTFMCEYADETATIVEWLNRWITFAQSIISTLTGGGGSGGGGSGGGGSEPKSSDKTHTCPPCPAPELLGGPSVFLFPPKPKDTLMISRTPEVTCVVVDVSHEDPEVKFNWYVDGVEVHNAKTKPREEQYGSTYRVVSVLTVLHQDWLNGKEYKCKVSNKALPAPIEKTISKAKGQPREPQVYTLPPSRDELTKNQVSLTCLVKGFYPSDIAVEWESNGQPENNYKTTPPVLDSDGSFFLYSKLTVDKSRWQQGNVFSCSVMHEALHNHYTQKSLSLSPGK

SEQ ID NO: 43 - protein, 380 aa, Artificial Sequence
APTSSSTKKTQLQLEELILDLQMILNGINNYKNPKLTRMLTFKFYMPKKATELKHLQCLEEELKPLEEVLNLAQSKNFHLRPRDLISNLNVIILELKGSETTFMCEYADETATIVEFLNRWITFAQSIISTLTGGGGSGGGGSGGGGSEPKSSDKTHTCPPCPAPELLGGPSVFLFPPKPKDTLMISRTPEVTCVVVDVSHEDPEVKFNWYVDGVEVHNAKTKPREEQYGSTYRVVSVLTVLHQDWLNGKEYKCKVSNKALPAPIEKTISKAKGQPREPQVYTLPPSRDELTKNQVSLTCLVKGFYPSDIAVEWESNGQPENNYKTTPPVLDSDGSFFLYSKLTVDKSRWQQGNVFSCSVMHEALHNHYTQKSLSLSPGK

SEQ ID NO: 44 - protein, 380 aa, Artificial Sequence
APTSSSTKKTQLQLEELLLDLQMILNWINNYKNPKLTRMLTFKFYMPKKATELKHLQCLEEELKPLEEVLNLAQSKNFHLRPRDLISNINVIVLELKGSETTFMCEYADETATIVEFLNFWITFAQSIISTLTGGGGSGGGGSGGGGSEPKSSDKTHTCPPCPAPELLGGPSVFLFPPKPKDTLMISRTPEVTCVVVDVSHEDPEVKFNWYVDGVEVHNAKTKPREEQYGSTYRVVSVLTVLHQDWLNGKEYKCKVSNKALPAPIEKTISKAKGQPREPQVYTLPPSRDELTKNQVSLTCLVKGFYPSDIAVEWESNGQPENNYKTTPPVLDSDGSFFLYSKLTVDKSRWQQGNVFSCSVMHEALHNHYTQKSLSLSPGK

SEQ ID NO: 45 - protein, 380 aa, Artificial Sequence
APTSSSTKKTQLQLEELLLDLQMILNGINNYKNPKLTRMLTFKFYMPKKATELKHLQCLEEELKPLEEVLNLAQSKNFHLRLRDLISNINVIVLELKGSETTFMCEYADETATIVEFLNFWITFAQSIISTLTGGGGSGGGGSGGGGSEPKSSDKTHTCPPCPAPELLGGPSVFLFPPKPKDTLMISRTPEVTCVVVDVSHEDPEVKFNWYVDGVEVHNAKTKPREEQYGSTYRVVSVLTVLHQDWLNGKEYKCKVSNKALPAPIEKTISKAKGQPREPQVYTLPPSRDELTKNQVSLTCLVKGFYPSDIAVEWESNGQPENNYKTTPPVLDSDGSFFLYSKLTVDKSRWQQGNVFSCSVMHEALHNHYTQKSLSLSPGK

SEQ ID NO: 46 - protein, 380 aa, Artificial Sequence
APTSSSTKKTQLQLEHLLLALQMILNGINNYKNPKLTRMLTFKFYMPKKATELKHLQCLEEELKPLEEVLNLAQSKNFHLRPRDLISNINVIVLELKGSETTFMCEYADETATIVEFLNRWITFAQSIISTLTGGGGSGGGGSGGGGSEPKSSDKTHTCPPCPAPELLGGPSVFLFPPKPKDTLMISRTPEVTCVVVDVSHEDPEVKFNWYVDGVEVHNAKTKPREEQYGSTYRVVSVLTVLHQDWLNGKEYKCKVSNKALPAPIEKTISKAKGQPREPQVYTLPPSRDELTKNQVSLTCLVKGFYPSDIAVEWESNGQPENNYKTTPPVLDSDGSFFLYSKLTVDKSRWQQGNVFSCSVMHEALHNHYTQKSLSLSPGK

SEQ ID NO: 47 - protein, 380 aa, Artificial Sequence
APTSSSTKKTQLQLEHLLLALQMILNGINNVKNPKLTRMLTFKFYMPKKATELKHLQCLEEELKPLEEVLNLLQSKNFQLRPRDLISNINVIVLELKGSETTFMCEYADETATIVEFLNRWITFAQSIISTLTGGGGSGGGGSGGGGSEPKSSDKTHTCPPCPAPELLGGPSVFLFPPKPKDTLMISRTPEVTCVVVDVSHEDPEVKFNWYVDGVEVHNAKTKPREEQYGSTYRVVSVLTVLHQDWLNGKEYKCKVSNKALPAPIEKTISKAKGQPREPQVYTLPPSRDELTKNQVSLTCLVKGFYPSDIAVEWESNGQPENNYKTTPPVLDSDGSFFLYSKLTVDKSRWQQGNVFSCSVMHEALHNHYTQKSLSLSPGK

SEQ ID NO: 48 - protein, 380 aa, Artificial Sequence
APTSSSTKKTQLQLEHLLLALQMILNGINNYKNPKLTRMLTFKFYMPKKATELKHLQCLEEELKPLEEVLNLAQSKNFHLRPRDLISNINVIVLELKGSETTFMCEYADETATIVEFLNFWITFAQSIISTLTGGGGSGGGGSGGGGSEPKSSDKTHTCPPCPAPELLGGPSVFLFPPKPKDTLMISRTPEVTCVVVDVSHEDPEVKFNWYVDGVEVHNAKTKPREEQYGSTYRVVSVLTVLHQDWLNGKEYKCKVSNKALPAPIEKTISKAKGQPREPQVYTLPPSRDELTKNQVSLTCLVKGFYPSDIAVEWESNGQPENNYKTTPPVLDSDGSFFLYSKLTVDKSRWQQGNVFSCSVMHEALHNHYTQKSLSLSPGK

SEQ ID NO: 49 - protein, 380 aa, Artificial Sequence
APTSSSTKKTQLQLEHLLLDLQMILNGINNYKNPKLTRMLTFKFYMPKKATELKHLQCLEEELKPLEEVLNLAQSKNFHLRPRDLISNINRIVLELKGSETTFMCEYADETATIVEFLNRWITFAQSIISTLTGGGGSGGGGSGGGGSEPKSSDKTHTCPPCPAPELLGGPSVFLFPPKPKDTLMISRTPEVTCVVVDVSHEDPEVKFNWYVDGVEVHNAKTKPREEQYGSTYRVVSVLTVLHQDWLNGKEYKCKVSNKALPAPIEKTISKAKGQPREPQVYTLPPSRDELTKNQVSLTCLVKGFYPSDIAVEWESNGQPENNYKTTPPVLDSDGSFFLYSKLTVDKSRWQQGNVFSCSVMHEALHNHYTQKSLSLSPGK

SEQ ID NO: 50 - protein, 380 aa, Artificial Sequence
APTSSSTKKTQLQLEHLLLDLQMILNGINNVKNPKLTRMLTFKFYMPKKATELKHLQCLEEELKPLEEVLNLLQSKNFQLRPRDLISNINRIVLELKGSETTFMCEYADETATIVEFLNRWITFAQSIISTLTGGGGSGGGGSGGGGSEPKSSDKTHTCPPCPAPELLGGPSVFLFPPKPKDTLMISRTPEVTCVVVDVSHEDPEVKFNWYVDGVEVHNAKTKPREEQYGSTYRVVSVLTVLHQDWLNGKEYKCKVSNKALPAPIEKTISKAKGQPREPQVYTLPPSRDELTKNQVSLTCLVKGFYPSDIAVEWESNGQPENNYKTTPPVLDSDGSFFLYSKLTVDKSRWQQGNVFSCSVMHEALHNHYTQKSLSLSPGK

SEQ ID NO: 51 - protein, 380 aa, Artificial Sequence
APTSSSTKKTQLLLEHLLLDLQMILNGINNYKNPKLTRMLTFKFYMPKKATELKHLQCLEEELKPLEEVLNLAQSKNFHLRPRDLISNINRIVLELKGSETTFMCEYADETATIVEFLNRWITFAQSIISTLTGGGGSGGGGSGGGGSEPKSSDKTHTCPPCPAPELLGGPSVFLFPPKPKDTLMISRTPEVTCVVVDVSHEDPEVKFNWYVDGVEVHNAKTKPREEQYGSTYRVVSVLTVLHQDWLNGKEYKCKVSNKALPAPIEKTISKAKGQPREPQVYTLPPSRDELTKNQVSLTCLVKGFYPSDIAVEWESNGQPENNYKTTPPVLDSDGSFFLYSKLTVDKSRWQQGNVFSCSVMHEALHNHYTQKSLSLSPGK

SEQ ID NO: 52 - protein, 380 aa, Artificial Sequence
APTSSSTKKTQLQLEHLLLDLQMILNGINNYKNPKLTRMLTFKFYMPKKATELKHLQCLEEELKPLEEVLNLAQSKNFHLRPRDLISNINRIVLELKGSETTFMCEYADETATIVEFLNFWITFAQSIISTLTGGGGSGGGGSGGGGSEPKSSDKTHTCPPCPAPELLGGPSVFLFPPKPKDTLMISRTPEVTCVVVDVSHEDPEVKFNWYVDGVEVHNAKTKPREEQYGSTYRVVSVLTVLHQDWLNGKEYKCKVSNKALPAPIEKTISKAKGQPREPQVYTLPPSRDELTKNQVSLTCLVKGFYPSDIAVEWESNGQPENNYKTTPPVLDSDGSFFLYSKLTVDKSRWQQGNVFSCSVMHEALHNHYTQKSLSLSPGK

SEQ ID NO: 53 - protein, 380 aa, Artificial Sequence
APTSSSTKKTQLQLEHLILDLQMILNGINNYKNPKLTRMLTFKFYMPKKATELKHLQCLEEELKPLEEVLNLAQSKNFHLRPRDLISNLNRIILELKGSETTFMCEYADETATIVEFLNRWITFAQSIISTLTGGGGSGGGGSGGGGSEPKSSDKTHTCPPCPAPELLGGPSVFLFPPKPKDTLMISRTPEVTCVVVDVSHEDPEVKFNWYVDGVEVHNAKTKPREEQYGSTYRVVSVLTVLHQDWLNGKEYKCKVSNKALPAPIEKTISKAKGQPREPQVYTLPPSRDELTKNQVSLTCLVKGFYPSDIAVEWESNGQPENNYKTTPPVLDSDGSFFLYSKLTVDKSRWQQGNVFSCSVMHEALHNHYTQKSLSLSPGK

SEQ ID NO: 54 - protein, 380 aa, Artificial Sequence
APTSSSTKKTQLQLEELLLDLQMILNGINNYKNPKLTRMLTFKFYMPKKATELKHLQCLEEELKPLEEVLNLAQSKNFHLRPRDLISNINRIVLELKGSETTFMCEYADETATIVEFLNRWITFAQSIISTLTGGGGSGGGGSGGGGSEPKSSDKTHTCPPCPAPELLGGPSVFLFPPKPKDTLMISRTPEVTCVVVDVSHEDPEVKFNWYVDGVEVHNAKTKPREEQYGSTYRVVSVLTVLHQDWLNGKEYKCKVSNKALPAPIEKTISKAKGQPREPQVYTLPPSRDELTKNQVSLTCLVKGFYPSDIAVEWESNGQPENNYKTTPPVLDSDGSFFLYSKLTVDKSRWQQGNVFSCSVMHEALHNHYTQKSLSLSPGK

SEQ ID NO: 55 - protein, 380 aa, Artificial Sequence
APTSSSTKKTQLQLEELLLDLQMILNGINNVKNPKLTRMLTFKFYMPKKATELKHLQCLEEELKPLEEVLNLLQSKNFQLRPRDLISNINRIVLELKGSETTFMCEYADETATIVEFLNRWITFAQSIISTLTGGGGSGGGGSGGGGSEPKSSDKTHTCPPCPAPELLGGPSVFLFPPKPKDTLMISRTPEVTCVVVDVSHEDPEVKFNWYVDGVEVHNAKTKPREEQYGSTYRVVSVLTVLHQDWLNGKEYKCKVSNKALPAPIEKTISKAKGQPREPQVYTLPPSRDELTKNQVSLTCLVKGFYPSDIAVEWESNGQPENNYKTTPPVLDSDGSFFLYSKLTVDKSRWQQGNVFSCSVMHEALHNHYTQKSLSLSPGK

SEQ ID NO: 56 - protein, 380 aa, Artificial Sequence
APTSSSTKKTQLQLEELILDLQMILNGINNYKNPKLTRMLTFKFYMPKKATELKHLQCLEEELKPLEEVLNLAQSKNFHLRPRDLISNLNRIILELKGSETTFMCEYADETATIVEFLNRWITFAQSIISTLTGGGGSGGGGSGGGGSEPKSSDKTHTCPPCPAPELLGGPSVFLFPPKPKDTLMISRTPEVTCVVVDVSHEDPEVKFNWYVDGVEVHNAKTKPREEQYGSTYRVVSVLTVLHQDWLNGKEYKCKVSNKALPAPIEKTISKAKGQPREPQVYTLPPSRDELTKNQVSLTCLVKGFYPSDIAVEWESNGQPENNYKTTPPVLDSDGSFFLYSKLTVDKSRWQQGNVFSCSVMHEALHNHYTQKSLSLSPGK

SEQ ID NO: 57 - protein, 272 aa, Homo sapiens
MDSYLLMWGLLTFIMVPGCQAELCDDDPPEIPHATFKAMAYKEGTMLNCECKRGFRRIKSGSLYMLCTGNSSHSSWDNQCQCTSSATRNTTKQVTPQPEEQKERKTTEMQSPMQPVDQASLPGHCREPPPWENEATERIYHFVVGQMVYYQCVQGYRALHRGPAESVCKMTHGKTRWTQPQLICTGEMETSQFPGEEKPQASPEGRPESETSCLVTTTDFQIQTEMAATMETSIFTTEYQVAVAGCVFLLISVLLLSGLTWQRRQRKSRRTI

SEQ ID NO: 58 - protein, 551 aa, Homo sapiens
MAAPALSWRLPLLILLLPLATSWASAAVNGTSQFTCFYNSRANISCVWSQDGALQDTSCQVHAWPDRRRWNQTCELLPVSQASWACNLILGAPDSQKLTTVDIVTLRVLCREGVRWRVMAIQDFKPFENLRLMAPISLQVVHVETHRCNISWEISQASHYFERHLEFEARTLSPGHTWEEAPLLTLKQKQEWICLETLTPDTQYEFQVRVKPLQGEFTTWSPWSQPLAFRTKPAALGKDTIPWLGHLLVGLSGAFGFIILVYLLINCRNTGPWLKKVLKCNTPDPSKFFSQLSSEHGGDVQKWLSSPFPSSSFSPGGLAPEISPLEVLERDKVTQLLLQQDKVPEPASLSSNHSLTSCFTNQGYFFFHLPDALEIEACQVYFTYDPYSEEDPDEGVAGAPTGSSPQPLQPLSGEDDAYCTFPSRDDLLLFSPSLLGGPSPPSTAPGGSGAGEERMPPSLQERVPRDWDPQPLGPPTPGVPDLVDFQPPPELVLREAGEEVPDAGPREGVSFPWSRPPGQGEFRALNARLPLNTDAYLSLQELQGQDPTHLV

SEQ ID NO: 59 - protein, 369 aa, Homo sapiens
MLKPSLPFTSLLFLQLPLLGVGLNTTILTPNGNEDTTADFFLTTMPTDSLSVSTLPLPEVQCFVFNVEYMNCTWNSSSEPQPTNLTLHYWYKNSDNDKVQKCSHYLFSEEITSGCQLQKKEIHLYQTFVVQLQDPREPRRQATQMLKLQNLVIPWAPENLTLHKLSESQLELNWNNRFLNHCLEHLVQYRTDWDHSWTEQSVDYRHKFSLPSVDGQKRYTFRVRSRFNPLCGSAQHWSEWSHPIHWGSNTSKENPFLFALEAVVISVGSMGLIISLLCVYFWLERTMPRIPTLKNLEDLVTEYHGNFSAWSGVSKGLAESLQPDYSERLCLVSEIPPKGGALGEGPGASPCNQHSPYWAPPCYTLKPET

SEQ ID NO: 60 - protein, 133 aa, Artificial Sequence
APTSSSTKKTQLQLEHLLLDLQMILNGINNYKNPKLTRMLTFKFYMPKKATELKHLQCLEEELKPLEEVLNLAQSKNFHLRPRDLISNINVIVLELKGSETTFMCEYADETATIVEFLNRWITFXQSIISTLT